European Patent Application EP 4 752 230 A1, published June 3, 2026. Title: METHODS FOR PRODUCING DNA PRODUCT. Applicant: 4basebio UK Ltd. The sequence listing filed with the application follows.

SEQUENCE LISTING (12 sequences)

SEQ ID NO: 1 - DNA, 85 bp, synthetic construct
  source 1..85: mol_type = other DNA
agggggagacgtaacatttgttggccactcatgggagggtgtgtggtcttggttggtgtgagtggccaacaaatgttacgtctcc

SEQ ID NO: 2 - DNA, 90 bp, synthetic construct
  source 1..90: mol_type = other DNA
agggggagacgtaacatttgttggccactcatcactttctacttatcgattaatcattggatgtgagtggccaacaaatgttacgtctcc

SEQ ID NO: 3 - DNA, 76 bp, synthetic construct
  source 1..76: mol_type = other DNA
agggggagacgtaacatttgttggccactcatatccacttttcaccatgtgagtggccaacaaatgttacgtctcc

SEQ ID NO: 4 - DNA, 24 bp, synthetic construct
  source 1..24: mol_type = other DNA
gggagggtgtgtggtcttggttgg

SEQ ID NO: 5 - DNA, 29 bp, synthetic construct
  source 1..29: mol_type = other DNA
cactttctacttatcgattaatcattgga

SEQ ID NO: 6 - DNA, 15 bp, synthetic construct
  source 1..15: mol_type = other DNA
atccacttttcacca

SEQ ID NO: 7 - DNA, 41 bp, synthetic construct
  source 1..41: mol_type = other DNA
agggctaacatttgttggccactcaggccaacaaatgttag

SEQ ID NO: 8 - DNA, 20 bp, synthetic construct
  source 1..20: mol_type = other DNA
  misc_feature 16..20: note = phosphorothioated nucleotide
aaaactaacatttgttggcc

SEQ ID NO: 9 - DNA, 16 bp, synthetic construct
  source 1..16: mol_type = other DNA
  misc_feature 1..5: note = phosphorothioated nucleotide
ggccaacaaatgttag

SEQ ID NO: 10 - DNA, 90 bp, synthetic construct
  source 1..90: mol_type = other DNA
aaaaggagacgtaacatttgttggccactcatcactttctacttatcgattaatcattggatgtgagtggccaacaaatgttacgtctcc

SEQ ID NO: 11 - DNA, 94 bp, synthetic construct
  source 1..94: mol_type = other DNA
nagggggagacgtaacatttgttggccactcatcactttctacttatcgattaatcattggatgagtggccaacaaatgttacgtctccccctn

SEQ ID NO: 12 - DNA, 92 bp, synthetic construct
  source 1..92: mol_type = other DNA
aaaaaggagacgtaacatttgttggccactcaggttactaattagctattcatctttcactgagtggccaacaaatgttacgtctccttttt